European Patent Specification EP 3 886 914 B1, published March 29, 2023. Title: ANTIBODY COMPRISING A GLUTAMINE-CONTAINING LIGHT CHAIN C-TERMINAL EXTENSION, CONJUGATES THEREOF, AND METHODS AND USES. Applicant: Bristol-Myers Squibb Company. The sequence listing filed with the application follows.

SEQUENCE LISTING (40 sequences)

SEQ ID NO: 1 - protein, 8 aa, Artificial Sequence
  C-Terminal Extension
GGVLQRAS

SEQ ID NO: 2 - protein, 8 aa, Artificial Sequence
  C-Terminal Extension
GGVLQGAS

SEQ ID NO: 3 - protein, 8 aa, Artificial Sequence
  C-Terminal Extension
GGVLQRPS

SEQ ID NO: 4 - protein, 8 aa, Artificial Sequence
  C-Terminal Extension
GGVLQGPS

SEQ ID NO: 5 - protein, 8 aa, Artificial Sequence
  C-Terminal Extension
GGVLQSPS

SEQ ID NO: 6 - protein, 8 aa, Artificial Sequence
  C-Terminal Extension
GGVLQYAS

SEQ ID NO: 7 - protein, 10 aa, Artificial Sequence
  C-Terminal Extension
GGGGVLQRAS

SEQ ID NO: 8 - protein, 10 aa, Artificial Sequence
  C-Terminal Extension
GGGGVLQGAS

SEQ ID NO: 9 - protein, 10 aa, Artificial Sequence
  C-Terminal Extension
GGGGVLQRPS

SEQ ID NO: 10 - protein, 10 aa, Artificial Sequence
  C-Terminal Extension
GGGGVLQGPS

SEQ ID NO: 11 - protein, 10 aa, Artificial Sequence
  C-Terminal Extension
GGGGVLQSPS

SEQ ID NO: 12 - protein, 10 aa, Artificial Sequence
  C-Terminal extension
GGGGVLQYAS

SEQ ID NO: 13 - protein, 6 aa, Artificial Sequence
  C-Terminal Extension
VLQYAS

SEQ ID NO: 14 - protein, 8 aa, Artificial Sequence
  C-Terminal Extension
GGVLQRQS

SEQ ID NO: 15 - protein, 8 aa, Artificial Sequence
  C-Terminal Extension
GGVLQGQS

SEQ ID NO: 16 - protein, 10 aa, Artificial Sequence
  C-Terminal Extension
GGVLQRQRPS

SEQ ID NO: 17 - protein, 10 aa, Artificial Sequence
  C-Terminal Extension
GGVLQGQGPS

SEQ ID NO: 18 - protein, 10 aa, Artificial Sequence
  C-Terminal Extension
GGVLQSQSPS

SEQ ID NO: 19 - protein, 8 aa, Artificial Sequence
  C-Terminal Extension
GGVLQYQS

SEQ ID NO: 20 - protein, 10 aa, Artificial Sequence
  C-Terminal extension
GGGGVLQRQS

SEQ ID NO: 21 - protein, 10 aa, Artificial Sequence
  C-Terminal Extension
GGGGVLQGQS

SEQ ID NO: 22 - protein, 12 aa, Artificial Sequence
  C-Terminal extension
GGGGVLQRQRPS

SEQ ID NO: 23 - protein, 12 aa, Artificial Sequence
  C-Terminal extension
GGGGVLQGQGPS

SEQ ID NO: 24 - protein, 12 aa, Artificial Sequence
  C-Terminal Extension
GGGGVLQSQSPS

SEQ ID NO: 25 - protein, 10 aa, Artificial Sequence
  C-Terminal Extension
GGGGVLQYQS

SEQ ID NO: 26 - protein, 6 aa, Artificial Sequence
  C-Terminal Extension
VLQYQS

SEQ ID NO: 27 - protein, 451 aa, Homo sapiens
  MISC_FEATURE: Anti-mesothelin antibody heavy chain
QVHLVESGGGVVQPGRSLRLSCVASGITFRIYGMHWVRQAPGKGLEWVAVLWYDGSHEYYADSVKGRFTISRDNSKNTLYLQMNSLRAEDTAIYYCARDGDYYDSGSPLDYWGQGTLVTVSSASTKGPSVFPLAPSSKSTSGGTAALGCLVKDYFPEPVTVSWNSGALTSGVHTFPAVLQSSGLYSLSSVVTVPSSSLGTQTYICNVNHKPSNTKVDKRVEPKSCDRTHTCPPCPAPELLGGPSVFLFPPKPKDTLMISRTPEVTCVVVDVSHEDPEVKFNWYVDGVEVHNAKTKPREEQYNSTYRVVSVLTVLHQDWLNGKEYKCKVSNKALPAPIEKTISKAKGQPREPQVYTLPPSREEMTKNQVSLTCLVKGFYPSDIAVEWESNGQPENNYKTTPPVLDSDGSFFLYSKLTVDKSRWQQGNVFSCSVMHEALHNHYTQKSLSLSPG

SEQ ID NO: 28 - protein, 214 aa, Homo sapiens
  MISC_FEATURE: Anti-mesothelin antibody kappa chain
EIVLTQSPATLSLSPGERATLSCRASQSVSSYLAWYQQKPGQAPRLLIYDASNRATGIPARFSGSGSGTDFTLTISSLEPEDFAVYYCQQRSNWPLTFGGGTKVEIKRTVAAPSVFIFPPSDEQLKSGTASVVCLLNNFYPREAKVQWKVDNALQSGNSQESVTEQDSKDSTYSLSSTLTLSKADYEKHKVYACEVTHQGLSSPVTKSFNRGEC

SEQ ID NO: 29 - protein, 9 aa, Artificial Sequence
  C-Terminal Extension
GGVLQVLQS

SEQ ID NO: 30 - protein, 10 aa, Artificial Sequence
  C-Terminal Extension
GGVLQGVLQS

SEQ ID NO: 31 - protein, 11 aa, Artificial Sequence
  C-Terminal Extension
GGVLQGGVLQS

SEQ ID NO: 32 - protein, 11 aa, Artificial Sequence
  C-Terminal Extension
GGVLQVLQGPS

SEQ ID NO: 33 - protein, 11 aa, Artificial Sequence
  C-Terminal Extension
GGVLQGGQGPS

SEQ ID NO: 34 - protein, 12 aa, Artificial Sequence
  C-Terminal Extension
GGVLQGGGQGPS

SEQ ID NO: 35 - protein, 11 aa, Artificial Sequence
  C-Terminal Extension
GGGGVLQVLQS

SEQ ID NO: 36 - protein, 12 aa, Artificial Sequence
  C-Terminal Extension
GGGGVLQGVLQS

SEQ ID NO: 37 - protein, 13 aa, Artificial Sequence
  C-Terminal Extension
GGGGVLQGGVLQS

SEQ ID NO: 38 - protein, 13 aa, Artificial Sequence
  C-Terminal Extension
GGGGVLQVLQGPS

SEQ ID NO: 39 - protein, 13 aa, Artificial Sequence
  C-Terminal Extension
GGGGVLQGGQGPS

SEQ ID NO: 40 - protein, 14 aa, Artificial Sequence
  C-Terminal Extension
GGGGVLQGGGQGPS